European Patent Application EP 4 144 759 A1, published March 8, 2023. Title: BISPECIFIC ANTIBODY TARGETING HUMAN CLAUDIN AND HUMAN PDL1 PROTEINS, AND APPLICATION THEREOF. Applicant: QURE BIOTECHNOLOGY (SHANGHAI) CO., LTD. The sequence listing filed with the application follows.

SEQUENCE LISTING (96 sequences)

SEQ ID NO: 1 - protein, 113 aa, Artificial Sequence
  Recombinant polypeptide
DIVMTQSPDSLAVSLGERATINCKSSQSLLNSGNQKNYLTWYQQKPGQPPKLLIYWASTRESGVPDRFSGSGSGTDFTLTISSLQAEDVAVYYCQNDYSYPFTFGQGTKLEIK

SEQ ID NO: 2 - protein, 113 aa, Artificial Sequence
  Recombinant polypeptide
DIVMTQSPDSLAVSLGERATISCKSSQSLLNSGNQKNYLTWYQQKPGQPPKLLIYWASTRESGVPDRFSGSGSGTDFTLTISSLQAEDVAVYYCQNDYSYPFTFGQGTKLEIK

SEQ ID NO: 3 - protein, 113 aa, Artificial Sequence
  Recombinant polypeptide
DIVMTQSPDSLAVSLGERATISCKSSQSLLNSGNQKNYLTWYQQKPGQPPKLLIYWASTRESGVPDRFTGSGSGTDFTLTISSLQAEDVAVYYCQNDYSYPFTFGQGTKLEIK

SEQ ID NO: 4 - protein, 117 aa, Artificial Sequence
  Recombinant polypeptide
EVQLVESGGGLVKPGGSLRLSCAASGFTFSNYAMSWVRQAPGKGLEWVSSIISGGRTYYLDSEKGRFTISRDNAKNSLYLQMNSLRAEDTAVYYCTRIYYGNSFDYWGQGTLVTVSS

SEQ ID NO: 5 - protein, 117 aa, Artificial Sequence
  Recombinant polypeptide
EVQLVESGGGLVKPGGSLRLSCAASGFTFSNYAMSWVRQAPGKGLEWVASIISGGRTYYLDSEKGRFTISRDNAKNSLYLQMNSLRAEDTAVYYCTRIYYGNSFDYWGQGTLVTVSS

SEQ ID NO: 6 - protein, 117 aa, Artificial Sequence
  Recombinant polypeptide
EVQLVESGGGLVKPGGSLRLSCAASGFTFSNYAMSWVRQAPGKRLEWVASIISGGRTYYLDSEKGRFTISRDNAKNSLYLQMNSLRAEDTAVYYCTRIYYGNSFDYWGQGTLVTVSS

SEQ ID NO: 7 - protein, 113 aa, Artificial Sequence
  Recombinant polypeptide
DIVMTQSPDSLAVSLGERATINCKSSQSLLNSGNQKNYLTWYQQKPGQPPKLLIYWASTRESGVPDRFSGSGSGTDFTLTISSLQAEDVAVYYCQNAYSYPFTFGQGTKLEIK

SEQ ID NO: 8 - protein, 113 aa, Artificial Sequence
  Recombinant polypeptide
DIVMTQSPDSLAVSLGERATISCKSSQSLLNSGNQKNYLTWYQQKPGQPPKLLIYWASTRESGVPDRFSGSGSGTDFTLTISSLQAEDVAVYYCQNAYSYPFTFGQGTKLEIK

SEQ ID NO: 9 - protein, 113 aa, Artificial Sequence
  Recombinant polypeptide
DIVMTQSPDSLAVSLGERATISCKSSQSLLNSGNQKNYLTWYQQKPGQPPKLLIYWASTRESGVPDRFSGSGSGIDFTLTISSVQAEDVAVYYCQNAYSYPFTFGQGTKLEIK

SEQ ID NO: 10 - protein, 113 aa, Artificial Sequence
  Recombinant polypeptide
DIVMTQSPDSLAVSLGERATISCKSSQSLLNSGNQKNYLTWYQQKPGQPPKMLIYWASTRESGVPDRFSGSGSGIDFTLTISSVQAEDVAVYYCQNAYSYPFTFGQGTKLEIK

SEQ ID NO: 11 - protein, 118 aa, Artificial Sequence
  Recombinant polypeptide
QVQLVQSGAEVKKPGASVKVSCKASGYAFSSYWMNWVRQAPGQGLEWMGQIYPGNGDTTYNGKFKGRVTMTRDTSTSTVYMELSSLRSEDTAVYYCARFVKGNAMDYWGQGTLVTVSS

SEQ ID NO: 12 - protein, 118 aa, Artificial Sequence
  Recombinant polypeptide
QVQLVQSGAEVKKPGASVKVSCKASGYAFSSYWMNWVRQAPGQGLEWIGQIYPGNGDTTYNGKFKGRVTMTADKSTSTVYMELSSLRSEDTAVYYCARFVKGNAMDYWGQGTLVTVSS

SEQ ID NO: 13 - protein, 118 aa, Artificial Sequence
  Recombinant polypeptide
QVQLVQSGAEVKKPGASVKVSCKASGYAFSSYWMNWVRQAPGQGLEWIGQIYPGNGDTTYNGKFKGRVTMTADKSTSTVYMELSSLRSEDTAVYFCARFVKGNAMDYWGQGTLVTVSS

SEQ ID NO: 14 - protein, 113 aa, Artificial Sequence
  Recombinant polypeptide
DIVMTQSPDSLAVSLGERATINCKSSQSLLNSGNQKNYLTWYQQKPGQPPKLLIYWASTRESGVPDRFSGSGSGTDFTLTISSLQAEDVAVYYCQNNYYYPLTFGGGTKVEIK

SEQ ID NO: 15 - protein, 113 aa, Artificial Sequence
  Recombinant polypeptide
DIVMTQSPDSLAVSLGERATISCKSSQSLLNSGNQKNYLTWYQQKPGQPPKLLIYWASTRESGVPDRFSGSGSGTDFTLTISSLQAEDVAVYFCQNNYYYPLTFGGGTKVEIK

SEQ ID NO: 16 - protein, 113 aa, Artificial Sequence
  Recombinant polypeptide
DIVMTQSPDSLAVSLGERATISCKSSQSLLNSGNQKNYLTWYQQKPGQPPKLLIYWASTRESGVPDRFTGSGSGTVFTLTISSLQAEDVAVYFCQNNYYYPLTFGGGTKVEIK

SEQ ID NO: 17 - protein, 119 aa, Artificial Sequence
  Recombinant polypeptide
EVQLVESGGGLVQPGGSLRLSCAASGFTFSSFGMHWVRQAPGKGLEWVSYISSGSNSIYYVDTVKGRFTISRDNAKNSLYLQMNSLRDEDTAVYYCARNAYYGNSFDYWGQGTLVTVSS

SEQ ID NO: 18 - protein, 119 aa, Artificial Sequence
  Recombinant polypeptide
EVQLVESGGGLVQPGGSLRLSCAASGFTFSSFGMHWVRQAPGKGLEWVAYISSGSNSIYYVDTVKGRFTISRDNAKNSLYLQMNSLRDEDTAVYYCARNAYYGNSFDYWGQGTLVTVSS

SEQ ID NO: 19 - protein, 119 aa, Artificial Sequence
  Recombinant polypeptide
EVQLVESGGGLVQPGGSLRLSCAASGFTFSSFGMHWVRQAPGKGLEWVAYISSGSNSIYYVDTVKGRFTISRDNAKNSLYLQMNSLRSEDTAVYYCARNAYYGNSFDYWGQGTLVTVSS

SEQ ID NO: 20 - protein, 113 aa, Artificial Sequence
  Recombinant polypeptide
DIVMTQSPDSLAVSLGERATINCKSSQSLLNSGNQKNYLTWYQQKPGQPPKLLIYWASTRESGVPDRFSGSGSGTDFTLTISSLQAEDVAVYYCQNDYSYPLTFGGGTKVEIK

SEQ ID NO: 21 - protein, 113 aa, Artificial Sequence
  Recombinant polypeptide
DIVMTQSPDSLAVSLGERATISCKSSQSLLNSGNQKNYLTWYQQKPGQAPKLLIYWASTRESGVPDRFSGSGSGTDFTLTISSLQAEDVAVYYCQNDYSYPLTFGGGTKVEIK

SEQ ID NO: 22 - protein, 113 aa, Artificial Sequence
  Recombinant polypeptide
DIVMTQSPDSLAVSLGERATISCKSSQSLLNSGNQKNYLTWYQQKPGQAPKLLIYWASTRESGVPDRFSGSGSGTDFTLTISSVQAEDVAVYFCQNDYSYPLTFGGGTKVEIK

SEQ ID NO: 23 - protein, 113 aa, Artificial Sequence
  Recombinant polypeptide
DIVMTQSPDSLAVSLGERATISCKSSQSLLNSGNQKNYLTWYQQKPGQAPKLLIYWASTRESGVPDRFIGSGSGTDFTLTISSVQAEDVAVYFCQNDYSYPLTFGGGTKVEIK

SEQ ID NO: 24 - protein, 115 aa, Artificial Sequence
  Recombinant polypeptide
QVQLVQSGAEVKKPGASVKVSCKASGYTFTNYFVHWVRQAPGQGLEWMGYINPYNDDTKYNEKFKGRVTMTRDTSTSTVYMELSSLRSEDTAVYYCLSLRFFAYWGQGTLVTVSS

SEQ ID NO: 25 - protein, 115 aa, Artificial Sequence
  Recombinant polypeptide
QVQLVQSGAEVKKPGASVKVSCKASGYTFTNYFVHWVRQAPGQGLEWIGYINPYNDDTKYNEKFKGRVTLTRDTSTSTVYMELSSLRSEDTAVYYCLSLRFFAYWGQGTLVTVSS

SEQ ID NO: 26 - protein, 115 aa, Artificial Sequence
  Recombinant polypeptide
QVQLVQSGAEVKKPGASVKVSCKASGYTFTNYFVHWVKQAPGQGLEWIGYINPYNDDTKYNEKFKGKATLTRDTSTSTVYMELSSLRSEDTAVYYCLSLRFFAYWGQGTLVTVSS

SEQ ID NO: 27 - protein, 115 aa, Artificial Sequence
  Recombinant polypeptide
QVQLVQSGAEVKKPGASVKVSCKASGYTFTNYFVHWVRQAPGQGLEWIGYINPYNDDTKYNEKFKGRVTLTSDKSTSTAYMELSSLRSEDTAVYYCLSLRFFAYWGQGTLVTVSS

SEQ ID NO: 28 - protein, 113 aa, Artificial Sequence
  Recombinant polypeptide
DIVMTQSPDSLAVSLGERATINCKSSQSLLNSGNQKNYLAWYQQKPGQPPKLLIYGASTRESGVPDRFSGSGSGTDFTLTISSLQAEDVAVYYCQNDHSYPFTFGQGTKLEIK

SEQ ID NO: 29 - protein, 113 aa, Artificial Sequence
  Recombinant polypeptide
DIVMTQSPDSLAVSLGERATINCKSSQSLLNSGNQKNYLAWYQQKPGQPPKLLIYGASTRESGVPDRFTGSGSGTDFTLTISSLQAEDVAVYYCQNDHSYPFTFGQGTKLEIK

SEQ ID NO: 30 - protein, 113 aa, Artificial Sequence
  Recombinant polypeptide
DIVMTQSPDSLAVSLGERATINCKSSQSLLNSGNQKNYLAWYQQKPGQPPKLLIYGASTRESGVPDRFTGSGSGTDFTLTISSVQAEDVAVYYCQNDHSYPFTFGQGTKLEIK

SEQ ID NO: 31 - protein, 120 aa, Artificial Sequence
  Recombinant polypeptide
QVQLVQSGAEVKKPGASVKVSCKASGYTFTSYIMHWVRQAPGQGLEWMGYINPYNDGTKYNEKFKGRVTMTRDTSTSTVYMELSSLRSEDTAVYYCARLGFTTRNAMDYWGQGTLVTVSS

SEQ ID NO: 32 - protein, 120 aa, Artificial Sequence
  Recombinant polypeptide
EVQLVQSGAEVKKPGASVKVSCKASGYTFTSYIMHWVRQAPGQGLEWIGYINPYNDGTKYNEKFKGRVTLTRDKSTSTVYMELSSLRSEDTAVYYCARLGFTTRNAMDYWGQGTLVTVSS

SEQ ID NO: 33 - protein, 120 aa, Artificial Sequence
  Recombinant polypeptide
EVQLVQSGAEVKKPGASVKVSCKASGYTFTSYIMHWVRQAPGQGLEWIGYINPYNDGTKYNEKFKGRVTLTSDKSTSTVYMELSSLRSEDTAVYYCARLGFTTRNAMDYWGQGTLVTVSS

SEQ ID NO: 34 - protein, 120 aa, Artificial Sequence
  Recombinant polypeptide
EVQLVQSGAEVKKPGASVKVSCKASGYTFTSYIMHWVKQAPGQGLEWIGYINPYNDGTKYNEKFKGKATLTSDKSTSTVYMELSSLRSEDTAVYCCARLGFTTRNAMDYWGQGTLVTVSS

SEQ ID NO: 35 - protein, 113 aa, Artificial Sequence
  Recombinant polypeptide
DIVMTQSPSSLTVTAGEKVTMSCKSSQSLLNSGNQKNYLTWYQQKPGQPPKLLIYWASTRESGVPDRFTGSGSGTDFTLTISSVQAEDLAVYYCQNDYSYPFTFGSGTKLEIK

SEQ ID NO: 36 - protein, 118 aa, Artificial Sequence
  Recombinant polypeptide
QVQLQQPGAELVRPGASVKLSCKASGYTFTSYWINWVKQRPGQGLEWIGNIYPSDSYTNYNQKFKDKATLTVDKSSSTAYMQLSSPTSEDSAVYYCTRSWRGNSFDYWGQGTTLTVSS

SEQ ID NO: 37 - protein, 113 aa, Artificial Sequence
  Recombinant polypeptide
DIVMTQSPSSQTVTAGEKVTMSCKSSQSLLNSGNQKNYLTWYQQKPGQPPKLLIYWASTRESGVPDRFTGSGSGTDFTLTISNMQAEDLAVYYCQNDYSYPFTFGSGTKLEIK

SEQ ID NO: 38 - protein, 117 aa, Mus musculus
EVKLVESGGGLVKPGGSLKLSCAASGFTFSNYAMSWVRQTPEKRLEWVASIISGGRTYYLDSEKGRFTISRDNARNNLYLQMSSLRSEDTAMYYCTRIYYGNSFDYWGQGTTLTVSS

SEQ ID NO: 39 - protein, 113 aa, Mus musculus
DIVMTQSPSSLTVTAGEKVTMSCKSSQSLLNSGNQKNYLTWYQQNPGQPPKMLIYWASTRESGVPDRFTGSGSGIDFSLTISSVQAEDLALYYCQNAYSYPFTFGSGTKLEIK

SEQ ID NO: 40 - protein, 118 aa, Mus musculus
QVQLQQSGAELVRPGSSVKISCKASGYAFSSYWMNWVKQRPGQGLEWIGQIYPGNGDTTYNGKFKGQATLTADKSSSTVYMQLSSLTSEDSAVYFCARFVKGNAMDYWGQGTSVTVSS

SEQ ID NO: 41 - protein, 113 aa, Mus musculus
DIVMTQSPSSLTVTAGEKVTMSCKSSQSLLNSGNQKNYLTWYQQKPGQPPKLLIYWASTRESGVPDRFTGSGSGTVFTLTISSVQAEDLAVYFCQNNYYYPLTFGAGTKLELK

SEQ ID NO: 42 - protein, 119 aa, Mus musculus
DVQLVESGGGLVQPGGSRKLSCAASGFTFSSFGMHWVRQAPEKGLEWVAYISSGSNSIYYVDTVKGRFTISRDNPKNTLFLQMTSLKSEDTAMYYCARNAYYGNSFDYWGQGTTLTVSS

SEQ ID NO: 43 - protein, 113 aa, Mus musculus
DIVMTQSPSSLTVTAGEKVTMSCKSSQSLLNSGNQKNYLTWYQQKPGQAPKLLIYWASTRESGVPDRFIGSGSGTDFTLTISHVQAEDLAVYFCQNDYSYPLTFGAGTNLELK

SEQ ID NO: 44 - protein, 115 aa, Mus musculus
EVQLQQSGPELVKPGASVKMSCKASGYTFTNYFVHWVKQKPGQGLEWIGYINPYNDDTKYNEKFKGKATLTSDKSSSTAYMDLSSLTSEDSAVYYCLSLRFFAYWGQGTLVTVSA

SEQ ID NO: 45 - protein, 113 aa, Mus musculus
DIVMTQSPSSLSVSAGEKVTMNCKSSQSLLNSGNQKNYLAWYQQKPGQPPKLLIYGASTRESGVPDRFTGSGSGTDFTLTISSVQAEDLAVYYCQNDHSYPFTFGSGTKLEIK

SEQ ID NO: 46 - protein, 120 aa, Mus musculus
EVQLQQSGPELVKPGASVKMSCKASGYTFTSYIMHWVKQKPGQGLEWIGYINPYNDGTKYNEKFKGKATLTSDKSSSTVYMELSSLTSEDSAVYCCARLGFTTRNAMDYWGQGTSVTVSS

SEQ ID NO: 47 - protein, 107 aa, Mus musculus
DIQMTQSPSTLSASVGDRVTITCRASQSISSWLAWYQQKPGKAPKLLIYDASSLESGVPSRFSGSGSGTEFTLTISSLQPDDFATYYCQQYNSYPLTFGQGTKVEIK

SEQ ID NO: 48 - protein, 120 aa, Mus musculus
EVQLLESGGGLVQPGGSLRLSCAASGFTFSSYAMSWVRQAPGKGLEWVSAISGSGGSTYYADSVKGRFTISRDNSKNTLYLQMNSLRAEDTAVYYCARDSYYYYFWYDYWGQGTLVTVSS

SEQ ID NO: 49 - protein, 126 aa, Mus musculus
EVQLLESGGGLVQPGGSLRLSCAASGFTYGTYAMSWVRQAPGKGLEWVSCIDIYGRASYTDPVKGRFTISRDNSKNTLYLQMNSLRAEDTAVYYCAARDFGYCTASWVHEGFSRYWGQGTLVTVSS

SEQ ID NO: 50 - protein, 126 aa, Mus musculus
EVQLLESGGGLVQPGGSLRLSCAASGFTYGTYAMSWVRQAPGKGLEWVACIDIYGRASYTDPVKGRFTISRDNSKNTLYLQMNSLKAEDTAVYYCAARDFGYCTASWVHEGFSRYWGQGTLVTVSS

SEQ ID NO: 51 - protein, 126 aa, Mus musculus
EVQLLESGGGLVQPGGSLRLSCAASGFTYGTYAMSWFRQAPGKGREGVACIDIYGRASYTDPVKGRFTISQDNSKNTLYLQMNSLKAEDTAVYYCAARDFGYCTASWVHEGFSRYWGQGTLVTVSS

SEQ ID NO: 52 - protein, 126 aa, Mus musculus
EVQLLESGGGLVQPGGSLRLSCAASGFTYGTYAMSWVRQAPGKGLEWVSCIDIYGRTSYTDPVKGRFTISRDNSKNTLYLQMNSLRAEDTAVYYCAARDFGYCTASWVHEGFSRYWGQGTLVTVSS

SEQ ID NO: 53 - protein, 126 aa, Mus musculus
EVQLLESGGGLVQPGGSLRLSCAASGFTYGTYAMSWVRQAPGKGLEWVACIDIYGRTSYTDPVKGRFTISQDNSKNTLYLQMNSLRAEDTAVYYCAARDFGYCTASWVHEGFSRYWGQGTLVTVSS

SEQ ID NO: 54 - protein, 126 aa, Mus musculus
EVQLLESGGGLVQPGGSLRLSCAASGFTYGTYAMSWFRQAPGKGLEGVACIDIYGRTSYTDPVKGRFTISQDNSKNTLYLQMNSLRAEDTAVYYCAARDFGYCTASWVHEGFSRYWGQGTLVTVSS

SEQ ID NO: 55 - protein, 126 aa, Camelus
QVQLVESGGGSVQSGGSLRLSCAASGFTYGTYAMSWFRQAPGKEREGVACIDIYGRASYTDPVKGRFTISQDNAKNTLYLQMNSLKPEDTAMYYCAARDFGYCTASWVHEGFSRYWGQGTQVTVSS

SEQ ID NO: 56 - protein, 126 aa, Camelus
QVQLVESGGDSVQPGGSLRLSCAASGFTYGTYAMSWFRQAPGKEREGVACIDIYGRTSYTDPVKGRFTISQDNAKNTLYLQMNSLKPEDTAMYYCAARDFGYCTASWVHEGFSRYWGQGTQVTVSS

SEQ ID NO: 57 - protein, 214 aa, Homo sapiens
DIQMTQSPSSLSASVGDRVTITCRASQDVSTAVAWYQQKPGKAPKLLIYSASFLYSGVPSRFSGSGSGTDFTLTISSLQPEDFATYYCQQYLYHPATFGQGTKVEIKRTVAAPSVFIFPPSDEQLKSGTASVVCLLNNFYPREAKVQWKVDNALQSGNSQESVTEQDSKDSTYSLSSTLTLSKADYEKHKVYACEVTHQGLSSPVTKSFNRGEC

SEQ ID NO: 58 - protein, 448 aa, Homo sapiens
EVQLVESGGGLVQPGGSLRLSCAASGFTFSDSWIHWVRQAPGKGLEWVAWISPYGGSTYYADSVKGRFTISADTSKNTAYLQMNSLRAEDTAVYYCARRHWPGGFDYWGQGTLVTVSSASTKGPSVFPLAPSSKSTSGGTAALGCLVKDYFPEPVTVSWNSGALTSGVHTFPAVLQSSGLYSLSSVVTVPSSSLGTQTYICNVNHKPSNTKVDKKVEPKSCDKTHTCPPCPAPELLGGPSVFLFPPKPKDTLMISRTPEVTCVVVDVSHEDPEVKFNWYVDGVEVHNAKTKPREEQYASTYRVVSVLTVLHQDWLNGKEYKCKVSNKALPAPIEKTISKAKGQPREPQVYTLPPSREEMTKNQVSLTCLVKGFYPSDIAVEWESNGQPENNYKTTPPVLDSDGSFFLYSKLTVDKSRWQQGNVFSCSVMHEALHNHYTQKSLSLSPGK

SEQ ID NO: 59 - protein, 220 aa, Artificial Sequence
  Recombinant polypeptide
DIVMTQSPDSLAVSLGERATINCKSSQSLLNSGNQKNYLTWYQQKPGQPPKLLIYWASTRESGVPDRFSGSGSGTDFTLTISSLQAEDVAVYYCQNDYSYPFTFGQGTKLEIKRTVAAPSVFIFPPSDEQLKSGTASVVCLLNNFYPREAKVQWKVDNALQSGNSQESVTEQDSKDSTYSLSSTLTLSKADYEKHKVYACEVTHQGLSSPVTKSFNRGEC

SEQ ID NO: 60 - protein, 592 aa, Artificial Sequence
  Recombinant polypeptide
EVQLVESGGGLVKPGGSLRLSCAASGFTFSNYAMSWVRQAPGKGLEWVASIISGGRTYYLDSEKGRFTISRDNAKNSLYLQMNSLRAEDTAVYYCTRIYYGNSFDYWGQGTLVTVSSASTKGPSVFPLAPSSKSTSGGTAALGCLVKDYFPEPVTVSWNSGALTSGVHTFPAVLQSSGLYSLSSVVTVPSSSLGTQTYICNVNHKPSNTKVDKKVEPKSCDKTHTCPPCPAPELLGGPSVFLFPPKPKDTLMISRTPEVTCVVVDVSHEDPEVKFNWYVDGVEVHNAKTKPREEQYNSTYRVVSVLTVLHQDWLNGKEYKCKVSNKALPAPIEKTISKAKGQPREPQVYTLPPSRDELTKNQVSLTCLVKGFYPSDIAVEWESNGQPENNYKTTPPVLDSDGSFFLYSKLTVDKSRWQQGNVFSCSVMHEALHNHYTQKSLSLSPGGGGGSGGGGSGGGGSGGGGSEVQLLESGGGLVQPGGSLRLSCAASGFTYGTYAMSWFRQAPGKGREGVACIDIYGRASYTDPVKGRFTISQDNSKNTLYLQMNSLKAEDTAVYYCAARDFGYCTASWVHEGFSRYWGQGTLVTVSS

SEQ ID NO: 61 - protein, 220 aa, Artificial Sequence
  Recombinant polypeptide
DIVMTQSPDSLAVSLGERATISCKSSQSLLNSGNQKNYLTWYQQKPGQPPKLLIYWASTRESGVPDRFSGSGSGTDFTLTISSLQAEDVAVYYCQNAYSYPFTFGQGTKLEIKRTVAAPSVFIFPPSDEQLKSGTASVVCLLNNFYPREAKVQWKVDNALQSGNSQESVTEQDSKDSTYSLSSTLTLSKADYEKHKVYACEVTHQGLSSPVTKSFNRGEC

SEQ ID NO: 62 - protein, 593 aa, Artificial Sequence
  Recombinant polypeptide
QVQLVQSGAEVKKPGASVKVSCKASGYAFSSYWMNWVRQAPGQGLEWIGQIYPGNGDTTYNGKFKGRVTMTADKSTSTVYMELSSLRSEDTAVYFCARFVKGNAMDYWGQGTLVTVSSASTKGPSVFPLAPSSKSTSGGTAALGCLVKDYFPEPVTVSWNSGALTSGVHTFPAVLQSSGLYSLSSVVTVPSSSLGTQTYICNVNHKPSNTKVDKKVEPKSCDKTHTCPPCPAPELLGGPSVFLFPPKPKDTLMISRTPEVTCVVVDVSHEDPEVKFNWYVDGVEVHNAKTKPREEQYNSTYRVVSVLTVLHQDWLNGKEYKCKVSNKALPAPIEKTISKAKGQPREPQVYTLPPSRDELTKNQVSLTCLVKGFYPSDIAVEWESNGQPENNYKTTPPVLDSDGSFFLYSKLTVDKSRWQQGNVFSCSVMHEALHNHYTQKSLSLSPGGGGGSGGGGSGGGGSGGGGSEVQLLESGGGLVQPGGSLRLSCAASGFTYGTYAMSWFRQAPGKGREGVACIDIYGRASYTDPVKGRFTISQDNSKNTLYLQMNSLKAEDTAVYYCAARDFGYCTASWVHEGFSRYWGQGTLVTVSS

SEQ ID NO: 63 - protein, 220 aa, Artificial Sequence
  Recombinant polypeptide
DIVMTQSPDSLAVSLGERATINCKSSQSLLNSGNQKNYLAWYQQKPGQPPKLLIYGASTRESGVPDRFTGSGSGTDFTLTISSLQAEDVAVYYCQNDHSYPFTFGQGTKLEIKRTVAAPSVFIFPPSDEQLKSGTASVVCLLNNFYPREAKVQWKVDNALQSGNSQESVTEQDSKDSTYSLSSTLTLSKADYEKHKVYACEVTHQGLSSPVTKSFNRGEC

SEQ ID NO: 64 - protein, 595 aa, Artificial Sequence
  Recombinant polypeptide
QVQLVQSGAEVKKPGASVKVSCKASGYTFTSYIMHWVRQAPGQGLEWMGYINPYNDGTKYNEKFKGRVTMTRDTSTSTVYMELSSLRSEDTAVYYCARLGFTTRNAMDYWGQGTLVTVSSASTKGPSVFPLAPSSKSTSGGTAALGCLVKDYFPEPVTVSWNSGALTSGVHTFPAVLQSSGLYSLSSVVTVPSSSLGTQTYICNVNHKPSNTKVDKKVEPKSCDKTHTCPPCPAPELLGGPSVFLFPPKPKDTLMISRTPEVTCVVVDVSHEDPEVKFNWYVDGVEVHNAKTKPREEQYNSTYRVVSVLTVLHQDWLNGKEYKCKVSNKALPAPIEKTISKAKGQPREPQVYTLPPSRDELTKNQVSLTCLVKGFYPSDIAVEWESNGQPENNYKTTPPVLDSDGSFFLYSKLTVDKSRWQQGNVFSCSVMHEALHNHYTQKSLSLSPGGGGGSGGGGSGGGGSGGGGSEVQLLESGGGLVQPGGSLRLSCAASGFTYGTYAMSWFRQAPGKGREGVACIDIYGRASYTDPVKGRFTISQDNSKNTLYLQMNSLKAEDTAVYYCAARDFGYCTASWVHEGFSRYWGQGTLVTVSS

SEQ ID NO: 65 - protein, 214 aa, Artificial Sequence
  Recombinant polypeptide
DIQMTQSPSTLSASVGDRVTITCRASQSISSWLAWYQQKPGKAPKLLIYDASSLESGVPSRFSGSGSGTEFTLTISSLQPDDFATYYCQQYNSYPLTFGQGTKVEIKRTVAAPSVFIFPPSDEQLKSGTASVVCLLNNFYPREAKVQWKVDNALQSGNSQESVTEQDSKDSTYSLSSTLTLSKADYEKHKVYACEVTHQGLSSPVTKSFNRGEC

SEQ ID NO: 66 - protein, 595 aa, Artificial Sequence
  Recombinant polypeptide
EVQLLESGGGLVQPGGSLRLSCAASGFTFSSYAMSWVRQAPGKGLEWVSAISGSGGSTYYADSVKGRFTISRDNSKNTLYLQMNSLRAEDTAVYYCARDSYYYYFWYDYWGQGTLVTVSSASTKGPSVFPLAPSSKSTSGGTAALGCLVKDYFPEPVTVSWNSGALTSGVHTFPAVLQSSGLYSLSSVVTVPSSSLGTQTYICNVNHKPSNTKVDKKVEPKSCDKTHTCPPCPAPELLGGPSVFLFPPKPKDTLMISRTPEVTCVVVDVSHEDPEVKFNWYVDGVEVHNAKTKPREEQYNSTYRVVSVLTVLHQDWLNGKEYKCKVSNKALPAPIEKTISKAKGQPREPQVYTLPPSRDELTKNQVSLTCLVKGFYPSDIAVEWESNGQPENNYKTTPPVLDSDGSFFLYSKLTVDKSRWQQGNVFSCSVMHEALHNHYTQKSLSLSPGGGGGSGGGGSGGGGSGGGGSEVQLLESGGGLVQPGGSLRLSCAASGFTYGTYAMSWFRQAPGKGREGVACIDIYGRASYTDPVKGRFTISQDNSKNTLYLQMNSLKAEDTAVYYCAARDFGYCTASWVHEGFSRYWGQGTLVTVSS

SEQ ID NO: 67 - protein, 107 aa, Homo sapiens [sequence omitted]

SEQ ID NO: 68 - protein, 330 aa, Homo sapiens [sequence omitted]

SEQ ID NO: 69 - protein, 5 aa, Camelus
TYAMS

SEQ ID NO: 70 - protein, 16 aa, Camelus
CIDIYGRASYTDPVKG

SEQ ID NO: 71 - protein, 19 aa, Camelus
ARDFGYCTASWVHEGFSRY

SEQ ID NO: 72 - protein, 17 aa, Mus musculus
KSSQSLLNSGNQKNYLT

SEQ ID NO: 73 - protein, 7 aa, Mus musculus
WASTRES

SEQ ID NO: 74 - protein, 9 aa, Mus musculus
QNDYSYPFT

SEQ ID NO: 75 - protein, 5 aa, Mus musculus
NYAMS

SEQ ID NO: 76 - protein, 16 aa, Mus musculus
SIISGGRTYYLDSEKG

SEQ ID NO: 77 - protein, 9 aa, Mus musculus
IYYGNSFDY

SEQ ID NO: 78 - protein, 9 aa, Mus musculus
QNAYSYPFT

SEQ ID NO: 79 - protein, 5 aa, Mus musculus
SYWMN

SEQ ID NO: 80 - protein, 17 aa, Mus musculus
QIYPGNGDTTYNGKFKG

SEQ ID NO: 81 - protein, 9 aa, Mus musculus
FVKGNAMDY

SEQ ID NO: 82 - protein, 9 aa, Mus musculus
QNNYYYPLT

SEQ ID NO: 83 - protein, 5 aa, Mus musculus
SFGMH

SEQ ID NO: 84 - protein, 17 aa, Mus musculus
YISSGSNSIYYVDTVKG

SEQ ID NO: 85 - protein, 10 aa, Mus musculus
NAYYGNSFDY

SEQ ID NO: 86 - protein, 9 aa, Mus musculus
QNDYSYPLT

SEQ ID NO: 87 - protein, 5 aa, Mus musculus
NYFVH

SEQ ID NO: 88 - protein, 17 aa, Mus musculus
YINPYNDDTKYNEKFKG

SEQ ID NO: 89 - protein, 8 aa, Mus musculus
LSLRFFAY

SEQ ID NO: 90 - protein, 17 aa, Mus musculus
KSSQSLLNSGNQKNYLA

SEQ ID NO: 91 - protein, 7 aa, Mus musculus
GASTRES

SEQ ID NO: 92 - protein, 9 aa, Mus musculus
QNDHSYPFT

SEQ ID NO: 93 - protein, 5 aa, Mus musculus
SYIMH

SEQ ID NO: 94 - protein, 17 aa, Mus musculus
YINPYNDGTKYNEKFKG

SEQ ID NO: 95 - protein, 11 aa, Mus musculus
LGFTTRNAMDY

SEQ ID NO: 96 - protein, 16 aa, Camelus
CIDIYGRTSYTDPVKG